European Patent Application EP 4 163 378 A1, published April 12, 2023. Title: Fusion protein of cytomegalovirus gB and pentamer and vaccine comprising the fusion protein. Applicant: KM Biologics Co., Ltd. The sequence listing filed with the application follows.

SEQUENCE LISTING (32 sequences)

SEQ ID NO: 1 - protein, 906 aa, Human cytomegalovirus
  HCMV AD169 gB
MESRIWCLVVCVNLCIVCLGAAVSSSSTSHATSSTHNGSHTSRTTSAQTRSVYSQHVTSSEAVSHRANETIYNTTLKYGDVVGVNTTKYPYRVCSMAQGTDLIRFERNIICTSMKPINEDLDEGIMVVYKRNIVAHTFKVRVYQKVLTFRRSYAYIYTTYLLGSNTEYVAPPMWEIHHINKFAQCYSSYSRVIGGTVFVAYHRDSYENKTMQLIPDDYSNTHSTRYVTVKDQWHSRGSTWLYRETCNLNCMLTITTARSKYPYHFFATSTGDVVYISPFYNGTNRNASYFGENADKFFIFPNYTIVSDFGRPNAAPETHRLVAFLERADSVISWDIQDEKNVTCQLTFWEASERTIRSEAEDSYHFSSAKMTATFLSKKQEVNMSDSALDCVRDEAINKLQQIFNTSYNQTYEKYGNVSVFETSGGLVVFWQGIKQKSLVELERLANRSSLNITHRTRRSTSDNNTTHLSSMESVHNLVYAQLQFTYDTLRGYINRALAQIAEAWCVDQRRTLEVFKELSKINPSAILSAIYNKPIAARFMGDVLGLASCVTINQTSVKVLRDMNVKESPGRCYSRPVVIFNFANSSYVQYGQLGEDNEILLGNHRTEECQLPSLKIFIAGNSAYEYVDYLFKRMIDLSSISTVDSMIALDIDPLENTDFRVLELYSQKELRSSNVFDLEEIMREFNSYKQRVKYVEDKVVDPLPPYLKGLDDLMSGLGAAGKAVGVAIGAVGGAVASVVEGVATFLKNPFGAFTIILVAIAVVIITYLIYTRQRRLCTQPLQNLFPYLVSADGTTVTSGSTKDTSLQAPPSYEESVYNSGRKGPGPPSSDASTAAPPYTNEQAYQMLLALARLDAEQRAQQNGTDSLDGQTGTQDKGQKPNLLDRLRHRKNGYRHLKDSDEEENV

SEQ ID NO: 2 - protein, 900 aa, Guinea pig cytomegalovirus
  GPCMV 22122 gB
MRPVRGIARSRILSCSWRGTWTSALTILYLGVYCESTTVTPTTVEDTTVSNGNHSDASRNNTVIRNLTASVDFSQRKLYPYRICSMSMGTDLVRFARTIQCVPFNPRVNSEEGIMLIYKRNILPYVFTAYTYQKELLFQRSYKYVTYDYLLGYSREFVALPMWEIFLVNSRGQCYTSHQRVIGADRYIAYHNDNEVNETMWLMRDDMGNDDTYRYITVKEHARTPGSVWLYKETCSMNCIVTKTKGKSKFPYDMFVLPSGVIVNISPFYNGSNGKTFREQREKFHIWSNYSILKDFGSRALEARIVPKMAFYEREDVVIGWEVNDQSNVTCEMILWETVDRAIRTEYENAFHYVARTLTSTFVENKYSPDNNLTEDDIKCFKNDAQKKIEEVFLRDYNETYDMDGNATYHVTTGGLVIVWQGLKQKSLKALEIAANESAVSATGSNSRRKRSLPDESTGDISYAQLQFAYDTLRTYINQALGHIAEAWCLDQKRTAEVLHELSKINPSNILSAIFGVPVAARVVGDVISLAKCIEVNQSTVLIKGDMRKFSDDGKLEGCYSRPVVWFSMKNSTEVRLGQLGEDNEILLGTHRMETCQTQDYRIFVAGDIGYEFQQYVFTKKINLSEIDIIDTMIALKTEPLENIDFKVLELYSRDELAQANVFDLESIMREYNYQKKRLDFVVERVINPIPPALKGLDEMMNGMGAIGKGIGEAVGAVGGAIGSFIGALVTFVTNPFGAFVVFLFCVGCITLVITVYRRQRRAMQRPFDYFFPYASQTITSSVADSSIAVAYPGPEGTSGDAPPPYPGEAPYGYKDLSVDADTRVSSSSAGAGADFNEEDAVRMLRAIKRLDDKKRQEIEKSSKDSASNKNSETRRRPGIMDRLRRRGGYQKLNTEDDVH

SEQ ID NO: 3 - protein, 682 aa, Human cytomegalovirus
  gB1-682-fm3Mv9
SSSTSHATSSTHNGSHTSRTTSAQTRSVYSQHVTSSEAVSHRANETIYNTTLKYGDVVGVNTTKYPYRVCSMAQGTDLIRFERNIICTSMKPINEDLDEGIMVVYKRNIVAHTFKVRVYQKVLTFRRSYAYHRTTYLLGSNTEYVAPPMWEIHHINKFAQCYSSYSRVIGGTVFVAYHRDSYENKTMQLIPDDYSNTHSTRYVTVKDQWHSRGSEALYRETCNLNCMLTITTARSKYPYHFFATSTGDVVYISPFYNGTNRNASYFGENADKFFIFPNYTIVSDFGRPNAAPETHRLVAFLERADSVISWDIQDEKNVTCQLTFWEASERTIRSEAEDSYHFSSAKMTATFLSKKQEVNMSDSALDCVRDEAINKLQQIFNTSYNQTYEKYGNVSVFETSGGLVVFWQGIKQKSLVELERLANRSSLNITHTTQRSTSDNNTTHLSSMESVHNLVYAQLQFTYDTLRGYINRALAQIAEAWCVDQRRTLEVFKELSKINPSAILSAIYNKPIAARFMGDVLGLASCVTINQTSVKVLRDMNVKESPGRCYSRPVVIFNFANSSYVQYGQLGEDNEILLGNHRTEECQLPSLKIFIAGNSAYEYVDYLFKRMIDLSSISTVDSMIALDIDPLENTDFRVLELYSQKELRSSNVFDLEEIMREFNSYKQRVKYVEDKVVDPLPP

SEQ ID NO: 4 - protein, 715 aa, Human cytomegalovirus
  gH ectodomain
MRPGLPSYLIILAVCLFSHLLSSRYGAEAVSEPLDKAFHLLLNTYGRPIRFLRENTTQCTYNSSLRNSTVVRENAISFNFFQSYNQYYVFHMPRCLFAGPLAEQFLNQVDLTETLERYQQRLNTYALVSKDLASYRSFSQQLKAQDSLGEQPTTVPPPIDLSIPHVWMPPQTTPHGWTESHTTSGLHRPHFNQTCILFDGHDLLFSTVTPCLHQGFYLIDELRYVKITLTEDFFVVTVSIDDDTPMLLIFGHLPRVLFKAPYQRDNFILRQTEKHELLVLVKKDQLNRHSYLKDPDFLDAALDFNYLDLSALLRNSFHRYAVDVLKSGRCQMLDRRTVEMAFAYALALFAAARQEEAGAQVSVPRALDRQAALLQIQEFMITCLSQTPPRTTLLLYPTAVDLAKRALWTPNQITDITSLVRLVYILSKQNQQHLIPQWALRQIADFALKLHKTHLASFLSAFARQELYLMGSLVHSMLVHTTERREIFIVETGLCSLAELSHFTQLLAHPHHEYLSDLYTPCSSSGRRDHSLERLTRLFPDATVPATVPAALSILSTMQPSTLETFPDLFCLPLGESFSALTVSEHVSYIVTNQYLIKGISYPVSTTVVGQSLIITQTDSQTKCELTRNMHTTHSITVALNISLENCAFCQSALLEYDDTQGVINIMYMHDSDDVLFALDPYNEVVVSSPRTHYLMLLKNGTVLEVTDVVVDATD

SEQ ID NO: 5 - protein, 278 aa, Human cytomegalovirus
  gL
MCRRPDCGFSFSPGPVILLWCCLLLPIVSSAAVSVAPTAAEKVPAECPELTRRCLLGEVFEGDKYESWLRPLVNVTGRDGPLSQLIRYRPVTPEAANSVLLDEAFLDTLALLYNNPDQLRALLTLLSSDTAPRWMTVMRGYSECGDGSPAVYTCVDDLCRGYDLTRLSYGRSIFTEHVLGFELVPPSLFNVVVAIRNEATRTNRAVRLPVSTAAAPEGITLFYGLYNAVKEFCLRHQLDPPLLRHLDKYYAGLPPELKQTRVNLPAHSRYGPQAVDAR

SEQ ID NO: 6 - protein, 171 aa, Human cytomegalovirus
  UL128
MSPKDLTPFLTALWLLLGHSRVPRVRAEECCEFINVNHPPERCYDFKMCNRFTVALRCPDGEVCYSPEKTAEIRGIVTTMTHSLTRQVVHNKLTSCNYNPLYLEADGRIRCGKVNDKAQYLLGAAGSVPYRWINLEYDKITRIVGLDQYLESVKKHKRLDVCRAKMGYMLQ

SEQ ID NO: 7 - protein, 214 aa, Human cytomegalovirus
  UL130
MLRLLLRHHFHCLLLCAVWATPCLASPWSTLTANQNPSPPWSKLTYSKPHDAATFYCPFLYPSPPRSPLQFSGFQRVSTGPECRNETLYLLYNREGQTLVERSSTWVKKVIWYLSGRNQTILQRMPRTASKPSDGNVQISVEDAKIFGAHMVPKQTKLLRFVVNDGTRYQMCVMKLESWAHVFRDYSVSFQVRLTFTEANNQTYTFCTHPNLIV

SEQ ID NO: 8 - protein, 129 aa, Human cytomegalovirus
  UL131
MRLCRVWLSVCLCAVVLGQCQRETAEKNDYYRVPHYWDACSRALPDQTRYKYVEQLVDLTLNYHYDASHGLDNFDVLKRINVTEVSLLISDFRRQNRRGGTNKRTTFNAAGSLAPHARSLEFSVRLFAN

SEQ ID NO: 9 - protein, 742 aa, Human cytomegalovirus
  gH
MRPGLPSYLIILAVCLFSHLLSSRYGAEAVSEPLDKAFHLLLNTYGRPIRFLRENTTQCTYNSSLRNSTVVRENAISFNFFQSYNQYYVFHMPRCLFAGPLAEQFLNQVDLTETLERYQQRLNTYALVSKDLASYRSFSQQLKAQDSLGEQPTTVPPPIDLSIPHVWMPPQTTPHGWTESHTTSGLHRPHFNQTCILFDGHDLLFSTVTPCLHQGFYLIDELRYVKITLTEDFFVVTVSIDDDTPMLLIFGHLPRVLFKAPYQRDNFILRQTEKHELLVLVKKDQLNRHSYLKDPDFLDAALDFNYLDLSALLRNSFHRYAVDVLKSGRCQMLDRRTVEMAFAYALALFAAARQEEAGAQVSVPRALDRQAALLQIQEFMITCLSQTPPRTTLLLYPTAVDLAKRALWTPNQITDITSLVRLVYILSKQNQQHLIPQWALRQIADFALKLHKTHLASFLSAFARQELYLMGSLVHSMLVHTTERREIFIVETGLCSLAELSHFTQLLAHPHHEYLSDLYTPCSSSGRRDHSLERLTRLFPDATVPATVPAALSILSTMQPSTLETFPDLFCLPLGESFSALTVSEHVSYIVTNQYLIKGISYPVSTTVVGQSLIITQTDSQTKCELTRNMHTTHSITVALNISLENCAFCQSALLEYDDTQGVINIMYMHDSDDVLFALDPYNEVVVSSPRTHYLMLLKNGTVLEVTDVVVDATDSRLLMMSVYALSAIIGIYLLYRMLKTC

SEQ ID NO: 10 - protein, 723 aa, Guinea pig cytomegalovirus
  GP75
MSPATRFTVISCLVVSLITPSETSSWFDPFIEWARSSPNMTCVNNRTGTRSLATEGLISFNFYEASRTVRTYQVPKCIFMSSVSKTIMQGVDLFESLESYRRRYYSYIIVPVHASFQIFIHDLRTDLSSPTEELTSPVDKTLPNVTIWHTPSGYVIRLLDVVTPRFEECTLFPNHTVIFDMTVPCSQEVYLRQTGKHQFAIVLTFTPSFFVLNIQTAQHQHVTENDEDVILIFGDVRSIDVKAPYSKPVLTLRQSYRDDLLIVAKTSIVNATYPFIKTQDFLKGTLSGNYLDFNHVYTEFNRLVIHNLVEGLCDAPPDDRTVSMVFSYAVLARTLYHTSNVTARLEDVALRYVRLTLARTFLQQCFDVGPRYMRFPTIDGALSVLLKLIRNSRDVDGGLKLSLTFALIFGNNTDMTKERDLENALYEMKSIHRAGLVSPLSPRQRSLLYMMAYVTHHTTAFPDIRREMLAMQTSLCSPQELYNWAPHVSSAGLTMQEMFTPCSGSGRRDYSEARIAEIVQLNPLTTKTPADLYRILAHFDRSNLTNFPALSCISHLSGYVAVTLRDVTYVVSSNVMLKGTSYPVTNLAVDKTMIVTVSPAQHPCEKTEVAHATRSIPIVKNITIGNDCEYCKSAIMEYDEVNGLSNIVYLADTADLVLVTNLDNRILASSPRTRYIMMTANGTLMEITSVIIDIRQTSIFMIMLYCSLGVLLLYGLYRLLHMI

SEQ ID NO: 11 - protein, 258 aa, Guinea pig cytomegalovirus
  GP115
MYECMFFSHRLTIGFYIPLIVLTTMSSLSESLGERQKTACTVAAISCANSDTYNRTTVSNHTFFYISDRWKYSELIRYEKPTGDLRHDKLIHVDREFLDIVSLLHNNENQLRTLLTIFRSDSAPPWVKFMRGYSQCLDHPIIYTCVEEKCQQYNLEELPYGKDIFLENVVGFDLGAPPHNMSVLIAVSNTKPKITKVLRITSTSLTLFDALYNTVLTFFRSIGARNVDVVRRLILYQASLSGPHRDAPIHNYLNRDLS

SEQ ID NO: 12 - protein, 179 aa, Guinea pig cytomegalovirus
  GP129
MRVIVLLVMFYYTRPGIFDDPCCIYSSKDRRVQHSTTSNDTWRLVRCGNTLMVAKRYTDSFCEFSLEENLFESLALNVSRQELHVLAPECKFGPVEVGINKQVRCIRYPRMPSVQSKPEKPSILGVTYRVDYTVMIPTPHFPRDFNGLLCTFLEKNDTFYNTTVDVCGSEFYSVDGNGK

SEQ ID NO: 13 - protein, 192 aa, Guinea pig cytomegalovirus
  GP131
MMKRYLVLLPWIMFYASFGRAGRCYYPSTPIPKSFVKHVDTTRSLPECENDTVAVLTLTNGAKLYVNMLNTWIDGYITTLQYAIPPTLSDIFAFIKRRIDYGSTGTAASTLPSLTSLRTYFGDRDSSFLWHYTIRMKDGAKTLDCDVYVTSRVHFVLNSYEAVQTVLFEGGVVISRHPADSIACLLINWNWT

SEQ ID NO: 14 - protein, 127 aa, Guinea pig cytomegalovirus
  GP133
MFWRLVYVYLVSLLLSIGAEDEGIDTWWLGGVTDNTRVKKENQLAHYILKTIVLTHHRRLRTGDECTEQLSNDLDIHSVHTLADSIRRLRGRYRKGLVSIDGIRISIQQSTRTQQKGLWISARIDRA

SEQ ID NO: 15 - protein, 682 aa, Human cytomegalovirus
  gB1-682
SSSTSHATSSTHNGSHTSRTTSAQTRSVYSQHVTSSEAVSHRANETIYNTTLKYGDVVGVNTTKYPYRVCSMAQGTDLIRFERNIICTSMKPINEDLDEGIMVVYKRNIVAHTFKVRVYQKVLTFRRSYAYIYTTYLLGSNTEYVAPPMWEIHHINKFAQCYSSYSRVIGGTVFVAYHRDSYENKTMQLIPDDYSNTHSTRYVTVKDQWHSRGSTWLYRETCNLNCMLTITTARSKYPYHFFATSTGDVVYISPFYNGTNRNASYFGENADKFFIFPNYTIVSDFGRPNAAPETHRLVAFLERADSVISWDIQDEKNVTCQLTFWEASERTIRSEAEDSYHFSSAKMTATFLSKKQEVNMSDSALDCVRDEAINKLQQIFNTSYNQTYEKYGNVSVFETSGGLVVFWQGIKQKSLVELERLANRSSLNITHRTRRSTSDNNTTHLSSMESVHNLVYAQLQFTYDTLRGYINRALAQIAEAWCVDQRRTLEVFKELSKINPSAILSAIYNKPIAARFMGDVLGLASCVTINQTSVKVLRDMNVKESPGRCYSRPVVIFNFANSSYVQYGQLGEDNEILLGNHRTEECQLPSLKIFIAGNSAYEYVDYLFKRMIDLSSISTVDSMIALDIDPLENTDFRVLELYSQKELRSSNVFDLEEIMREFNSYKQRVKYVEDKVVDPLPP

SEQ ID NO: 16 - protein, 433 aa, Human cytomegalovirus
  gB delta d4
LDEGIMVVYKRNIVAHTFKVRVYQKVLTFRRSYAAAATTYLLGSNTEYVAPPMWEIHHINKFAQCYSSYSRVIGGTVFVAYHRDSYENKTMQLIPDDYSNTHSTRYVTVKDQWHSRGSTALYRETCNLNCMLTITTARSKYPYHFFATSTGDVVYISPFYNGTNRNASYFGENADKFFIFPNYTIVSDFGRPNAAPETHRLVAFLERADSVISWDIQDEKNVTCQLTFWEASERTIRSEAEDSYHFSSAKMTATFLSKKQEVNMSDSALDCVRDEAINKLQQIFNTSYNQTYEKYGNVSVFETSGGLVVFWQGIKQKSLVELERLANRSSLNITHTTQRSTSDNNTTHLSSMESVHNLVYAQLQFTYDTLRGGGGSGSGGGLENTDFRVLELYSQKELRSSNVFDLEEIMREFNSYKQRVKYVEDKVVDPLPP

SEQ ID NO: 17 - protein, 692 aa, Guinea pig cytomegalovirus
  GPCMV gB ectodomain
MRPVRGIARSRILSCSWRGTWTSALTILYLGVYCESTTVTPTTVEDTTVSNGNHSDASRNNTVIRNLTASVDFSQRKLYPYRICSMSMGTDLVRFARTIQCVPFNPRVNSEEGIMLIYKRNILPYVFTAYTYQKELLFQRSYKGHRYDYLLGYSREFVALPMWEIFLVNSRGQCYTSHQRVIGADRYIAYHNDNEVNETMWLMRDDMGNDDTYRYITVKEHARTPGSVAFHKETCSMNCIVTKTKGKSKFPYDMFVLPSGVIVNISPFYNGSNGKTFREQREKFHIWSNYSILKDFGSRALEARIVPKMAFYEREDVVIGWEVNDQSNVTCEMILWETVDRAIRTEYENAFHYVARTLTSTFVENKYSPDNNLTEDDIKCFKNDAQKKIEEVFLRDYNETYDMDGNATYHVTTGGLVIVWQGLKQKSLKALEIAANESAVSATGSNSRRKRSLPDESTGDISYAQLQFAYDTLRTYINQALGHIAEAWCLDQKRTAEVLHELSKINPSNILSAIFGVPVAARVVGDVISLAKCIEVNQSTVLIKGDMRKFSDDGKLEGCYSRPVVWFSMKNSTEVRLGQLGEDNEILLGTHRMETCQTQDYRIFVAGDIGYEFQQYVFTKKINLSEIDIIDTMIALKTEPLENIDFKVLELYSRDELAQANVFDLESIMREYNYQKKRLDFVVERVINPIPP

SEQ ID NO: 18 - protein, 698 aa, Guinea pig cytomegalovirus
  GP75 ectodomain
MSPATRFTVISCLVVSLITPSETSSWFDPFIEWARSSPNMTCVNNRTGTRSLATEGLISFNFYEASRTVRTYQVPKCIFMSSVSKTIMQGVDLFESLESYRRRYYSYIIVPVHASFQIFIHDLRTDLSSPTEELTSPVDKTLPNVTIWHTPSGYVIRLLDVVTPRFEECTLFPNHTVIFDMTVPCSQEVYLRQTGKHQFAIVLTFTPSFFVLNIQTAQHQHVTENDEDVILIFGDVRSIDVKAPYSKPVLTLRQSYRDDLLIVAKTSIVNATYPFIKTQDFLKGTLSGNYLDFNHVYTEFNRLVIHNLVEGLCDAPPDDRTVSMVFSYAVLARTLYHTSNVTARLEDVALRYVRLTLARTFLQQCFDVGPRYMRFPTIDGALSVLLKLIRNSRDVDGGLKLSLTFALIFGNNTDMTKERDLENALYEMKSIHRAGLVSPLSPRQRSLLYMMAYVTHHTTAFPDIRREMLAMQTSLCSPQELYNWAPHVSSAGLTMQEMFTPCSGSGRRDYSEARIAEIVQLNPLTTKTPADLYRILAHFDRSNLTNFPALSCISHLSGYVAVTLRDVTYVVSSNVMLKGTSYPVTNLAVDKTMIVTVSPAQHPCEKTEVAHATRSIPIVKNITIGNDCEYCKSAIMEYDEVNGLSNIVYLADTADLVLVTNLDNRILASSPRTRYIMMTANGTLMEITSVIIDIRQTS

SEQ ID NO: 19 - protein, 24 aa, Human cytomegalovirus
  HCMV gB signal sequence
MESRIWCLVVCVNLCIVCLGAAVS

SEQ ID NO: 20 - protein, 9 aa, Artificial Sequence
  9 amino acid linker
GGGSGSGGG

SEQ ID NO: 21 - protein, 20 aa, Homo sapiens
  Immonoglobulin light chain signal peptide sequence
MRLPAQLLGLLMLWVPGSSG

SEQ ID NO: 22 - protein, 5 aa, Artificial Sequence
  5 amino acids linker
GGGGS

SEQ ID NO: 23 - protein, 15 aa, Artificial Sequence
  15 amino acids linker
GGGGSGGGGSGGGGS

SEQ ID NO: 24 - DNA, 22 bp, Artificial Sequence
  GPCMV GP83 Forward Primer
cgacgacgacgatgacgaaaac

SEQ ID NO: 25 - DNA, 22 bp, Artificial Sequence
  GPCMV GP83 Reverse Primer
tcctcggtctcaacgaagggtc

SEQ ID NO: 26 - DNA, 17 bp, Artificial Sequence
  GPCMV GP83 FAM Probe
atccgagttaggcagcg

SEQ ID NO: 27 - DNA, 17 bp, Artificial Sequence
  Guinea pigs beta-actin Forward Primer
tggatcggcggctcatc

SEQ ID NO: 28 - DNA, 22 bp, Artificial Sequence
  Guinea pigs beta-actin Reverse Primer
catcgtactcctgcttgctgat

SEQ ID NO: 29 - DNA, 15 bp, Artificial Sequence
  Guinea pigs beta-actin Probe
cactctccaccttcc

SEQ ID NO: 30 - protein, 9 aa, Artificial Sequence
  His tag
LGGHHHHHH

SEQ ID NO: 31 - protein, 671 aa, Human cytomegalovirus
  gBVC37
SSSTSHATSSTHNGSHTSRTTSAQTRSVYSQHVTSSEAVSHRANETIYNTTLKYGDVVGVNTTKYPYRVCSMAQGTNLTRFERNIICTSMKPINEDLDEGIMVVYKRNIVAHTFKVRVYQKVLTFRRGGGGSNTEYVAPPMWEIHHINKFAQCYSSYSRVIGGTVFVAYHRDSYENKTMQLIPDDYSNTHSTRYVTVKDQWHSRGSERETCNLNCMLTITTARSKYPYHFFATSTGDVVYISPFYNGTNRNASYFGENADKFFIFPNYTIVSDFGRPNAAPETHRLVAFLERADSVISWDIQDEKNVTCQLTFWEASERTIRSEAEDSYHFSSAKMTATFLSKKQEVNMSDSALDCVRDEAINKLQQIFNTSYNQTYEKYGNVSVFETSGGLVVFWQGIKQKSLVELERLANRSSLNITHTTQRSTSDNNTTHLSSMESVHNLVYAQLQFTYDTLRGYINRALAQIAEAWCVDQRRTLEVFKELSKINPSAILSAIYNKPIAARFMGDVLGLASCVTINQTSVKVLRDMNVKNSTGRCYSRPVVIFNFANSSYVQYGQLGEDNEILLGNHRTEECQNGSLKIFIAGNSAYEYVDYLFNTTIDLSSISTVDSMIALDIDPLENTDFRVLELYSQKELRSSNVFDLEEIMREFNSYKQRVKYVEDKVVDPLPP

SEQ ID NO: 32 - protein, 435 aa, Guinea pig cytomegalovirus
  GPCMV-gB delta d4
EEGIMLIYKRNILPYVFTAYTYQKELLFQRSYKGHRYDYLLGYSREFVALPMWEIFLVNSRGQCYTSHQRVIGADRYIAYHNDNEVNETMWLMRDDMGNDDTYRYITVKEHARTPGSVAFHKETCSMNCIVTKTKGKSKFPYDMFVLPSGVIVNISPFYNGSNGKTFREQREKFHIWSNYSILKDFGSRALEARIVPKMAFYEREDVVIGWEVNDQSNVTCEMILWETVDRAIRTEYENAFHYVARTLTSTFVENKYSPDNNLTEDDIKCFKNDAQKKIEEVFLRDYNETYDMDGNATYHVTTGGLVIVWQGLKQKSLKALEIAANESAVSATGSNSRRKRSLPDESTGDISYAQLQFAYDTLRTGGGSGSGGGLENIDFKVLELYSRDELAQANVFDLESIMREYNYQKKRLDFVVERVINPIPPLGGHHHHHH